European Patent Application EP 4 644 406 A1, published November 5, 2025. Title: 放射性標識医薬. Applicant: 国立大学法人千葉大学. The sequence listing filed with the application follows.

SEQUENCE LISTING (3 sequences)

SEQ ID NO: 1 - protein, 5 aa, synthetic construct
  CROSSLNK 1..5: note = Lysyl Arginine Peptide (Lys-Arg)
  SITE 4: note = D-Phenylalanine
RGDFK

SEQ ID NO: 2 - protein, 9 aa, synthetic construct
  SITE 3: note = Norleucine
  SITE 6: note = D-Phenylalanine
  CROSSLNK 4..9: note = (3-amino-3-carboxypropanoyl)Arginine Peptide (Lys-Asp)
GGXDHFRWK

SEQ ID NO: 3 - protein, 8 aa, synthetic construct
  SITE 1: note = D-Phenylalanine
  SITE 4: note = D-Tryptophan
  DISULFID 2..7: note = Cys-Cys
FCYWKTCT